European Patent Specification EP 3 579 860 B1, published November 12, 2025. Title: TRAILshort ANTIBODY AND METHODS OF USE. Applicant: Mayo Foundation for Medical Education and Research. The sequence listing filed with the application follows.

SEQUENCE LISTING (31 sequences)

SEQ ID NO: 1 - protein, 10 aa, Artificial Sequence
  TRAILshort antibody VH CDR1 domain
GYIFTNNDMN

SEQ ID NO: 2 - protein, 17 aa, Artificial Sequence
  TRAILshort antibody VH CDR2 domain
GIDPGDGRTKYNEKFKG

SEQ ID NO: 3 - protein, 11 aa, Artificial Sequence
  TRAILshort antibody VH CDR3 domain
GRGGYEFGIDY

SEQ ID NO: 4 - protein, 118 aa, Artificial Sequence
  TRAILshort antibody VH domain
QVQLQQSGPELVKPGASVKISCKASGYIFTNNDMNWVKQRPGQGLEWIGGIDPGDGRTKYNEKFKGKATLTADKFSNTVYMQLSSLTSENSAVYFCGRGGYEFGIDYWGQGTSVTVSS

SEQ ID NO: 5 - protein, 118 aa, Artificial Sequence
  TRAILshort antibody VH domain
QVQLVQSGAEVKKPGATVKISCKVSGYIFTNNDMNWVQQAPGKGLEWMGGIDPGDGRTKYNEKFKGRVTITADESTSTAYMELSSLRSEDTAVYYCGRGGYEFGIDYWGQGTLVTVSS

SEQ ID NO: 6 - protein, 118 aa, Artificial Sequence
  TRAILshort antibody VH domain
QVQLVQSGAEVKKPGASVKVSCKASGYIFTNNDMNWVRQAPGQGLEWMGGIDPGDGRTKYNEKFKGRVTMTRDTSTNTVYMELSSLTSEDTAVYFCGRGGYEFGIDYWGQGTTVTVSS

SEQ ID NO: 7 - protein, 118 aa, Artificial Sequence
  TRAILshort antibody VH domain
QVQLVQSGAEVKKPGSSVKVSCKSSGYIFTNNDMNWVRQAPGQGLDWMGGIDPGDGRTKYNEKFKGRVTISADIFSNTAYMELNSLTSEDTAVYFCGRGGYEFGIDYWGQGTTVTVSS

SEQ ID NO: 8 - protein, 118 aa, Artificial Sequence
  TRAILshort antibody VH domain
QVQLVESGAEVKKPGASVKVSCKVSGYIFTNNDMNWVRQAPGEGLEWMGGIDPGDGRTKYNEKFKGRVTMTEDTSTDTAYMELSSLRSEDTAVYYCGRGGYEFGIDYWGQGTTVTVSS

SEQ ID NO: 9 - protein, 467 aa, Artificial Sequence
  TRAILshort antibody heavy chain
MGWTLVFLFLLSVTAGVHSQVQLQQSGPELVKPGASVKISCKASGYIFTNNDMNWVKQRPGQGLEWIGGIDPGDGRTKYNEKFKGKATLTADKFSNTVYMQLSSLTSENSAVYFCGRGGYEFGIDYWGQGTSVTVSSASTKGPSVFPLAPSSKSTSGGTAALGCLVKDYFPEPVTVSWNSGALTSGVHTFPAVLQSSGLYSLSSVVTVPSSSLGTQTYICNVNHKPSNTKVDKKVEPKSCDKTHTCPPCPAPELLGGPSVFLFPPKPKDTLMISRTPEVTCVVVDVSHEDPEVKFNWYVDGVEVHNAKTKPREEQYNSTYRVVSVLTVLHQDWLNGKEYKCKVSNKALPAPIEKTISKAKGQPREPQVYTLPPSRDELTKNQVSLTCLVKGFYPSDIAVEWESNGQPENNYKTTPPVLDSDGSFFLYSKLTVDKSRWQQGNVFSCSVMHEALHNHYTQKSLSLSPGK

SEQ ID NO: 10 - protein, 467 aa, Artificial Sequence
  TRAILshort antibody heavy chain
MGWTLVFLFLLSVTAGVHSQVQLVQSGAEVKKPGATVKISCKVSGYIFTNNDMNWVQQAPGKGLEWMGGIDPGDGRTKYNEKFKGRVTITADESTSTAYMELSSLRSEDTAVYYCGRGGYEFGIDYWGQGTLVTVSSASTKGPSVFPLAPSSKSTSGGTAALGCLVKDYFPEPVTVSWNSGALTSGVHTFPAVLQSSGLYSLSSVVTVPSSSLGTQTYICNVNHKPSNTKVDKKVEPKSCDKTHTCPPCPAPELLGGPSVFLFPPKPKDTLMISRTPEVTCVVVDVSHEDPEVKFNWYVDGVEVHNAKTKPREEQYNSTYRVVSVLTVLHQDWLNGKEYKCKVSNKALPAPIEKTISKAKGQPREPQVYTLPPSRDELTKNQVSLTCLVKGFYPSDIAVEWESNGQPENNYKTTPPVLDSDGSFFLYSKLTVDKSRWQQGNVFSCSVMHEALHNHYTQKSLSLSPGK

SEQ ID NO: 11 - protein, 467 aa, Artificial Sequence
  TRAILshort antibody heavy chain
MGWTLVFLFLLSVTAGVHSQVQLVQSGAEVKKPGASVKVSCKASGYIFTNNDMNWVRQAPGQGLEWMGGIDPGDGRTKYNEKFKGRVTMTRDTSTNTVYMELSSLTSEDTAVYFCGRGGYEFGIDYWGQGTTVTVSSASTKGPSVFPLAPSSKSTSGGTAALGCLVKDYFPEPVTVSWNSGALTSGVHTFPAVLQSSGLYSLSSVVTVPSSSLGTQTYICNVNHKPSNTKVDKKVEPKSCDKTHTCPPCPAPELLGGPSVFLFPPKPKDTLMISRTPEVTCVVVDVSHEDPEVKFNWYVDGVEVHNAKTKPREEQYNSTYRVVSVLTVLHQDWLNGKEYKCKVSNKALPAPIEKTISKAKGQPREPQVYTLPPSRDELTKNQVSLTCLVKGFYPSDIAVEWESNGQPENNYKTTPPVLDSDGSFFLYSKLTVDKSRWQQGNVFSCSVMHEALHNHYTQKSLSLSPGK

SEQ ID NO: 12 - protein, 467 aa, Artificial Sequence
  TRAILshort antibody heavy chain
MGWTLVFLFLLSVTAGVHSQVQLVQSGAEVKKPGSSVKVSCKSSGYIFTNNDMNWVRQAPGQGLDWMGGIDPGDGRTKYNEKFKGRVTISADIFSNTAYMELNSLTSEDTAVYFCGRGGYEFGIDYWGQGTTVTVSSASTKGPSVFPLAPSSKSTSGGTAALGCLVKDYFPEPVTVSWNSGALTSGVHTFPAVLQSSGLYSLSSVVTVPSSSLGTQTYICNVNHKPSNTKVDKKVEPKSCDKTHTCPPCPAPELLGGPSVFLFPPKPKDTLMISRTPEVTCVVVDVSHEDPEVKFNWYVDGVEVHNAKTKPREEQYNSTYRVVSVLTVLHQDWLNGKEYKCKVSNKALPAPIEKTISKAKGQPREPQVYTLPPSRDELTKNQVSLTCLVKGFYPSDIAVEWESNGQPENNYKTTPPVLDSDGSFFLYSKLTVDKSRWQQGNVFSCSVMHEALHNHYTQKSLSLSPGK

SEQ ID NO: 13 - protein, 467 aa, Artificial Sequence
  TRAILshort antibody heavy chain
MGWTLVFLFLLSVTAGVHSQVQLVESGAEVKKPGASVKVSCKVSGYIFTNNDMNWVRQAPGEGLEWMGGIDPGDGRTKYNEKFKGRVTMTEDTSTDTAYMELSSLRSEDTAVYYCGRGGYEFGIDYWGQGTTVTVSSASTKGPSVFPLAPSSKSTSGGTAALGCLVKDYFPEPVTVSWNSGALTSGVHTFPAVLQSSGLYSLSSVVTVPSSSLGTQTYICNVNHKPSNTKVDKKVEPKSCDKTHTCPPCPAPELLGGPSVFLFPPKPKDTLMISRTPEVTCVVVDVSHEDPEVKFNWYVDGVEVHNAKTKPREEQYNSTYRVVSVLTVLHQDWLNGKEYKCKVSNKALPAPIEKTISKAKGQPREPQVYTLPPSRDELTKNQVSLTCLVKGFYPSDIAVEWESNGQPENNYKTTPPVLDSDGSFFLYSKLTVDKSRWQQGNVFSCSVMHEALHNHYTQKSLSLSPGK

SEQ ID NO: 14 - protein, 17 aa, Artificial Sequence
  TRAILshort antibody VL CDR1 domain
KSSQSLLNSGNQKNSLA

SEQ ID NO: 15 - protein, 7 aa, Artificial Sequence
  TRAILshort antibody VL CDR2 domain
GASTRES

SEQ ID NO: 16 - protein, 9 aa, Artificial Sequence
  TRAILshort antibody VL CDR3 domain
QNDHSFPLT

SEQ ID NO: 17 - protein, 113 aa, Artificial Sequence
  TRAILshort antibody VL domain
DIVMTQSPSSLSVSAGEKVTMSCKSSQSLLNSGNQKNSLAWYQQKPGRPPTLLISGASTRESGVPDRFTGSGSGTDFTLTISSVQAEDLAVYYCQNDHSFPLTFGAGTKLELK

SEQ ID NO: 18 - protein, 113 aa, Artificial Sequence
  TRAILshort antibody VL domain
DVVMTQSPDSLAVSLGERATINCKSSQSLLNSGNQKNSLAWYQQKPGQPPKLLIYGASTRESGVPDRFSGSGSGTDFTLTISSLQAEDVAVYYCQNDHSFPLTFGQGTKLEIK

SEQ ID NO: 19 - protein, 113 aa, Artificial Sequence
  TRAILshort antibody VL domain
DIVMTQSPDSLAVSLGERATINCKSSQSLLNSGNQKNSLAWYQQKPGQPPKLLIYGASTRESGVPDRFSGSGSGTDFTLTISSLQAEDVAVYYCQNDHSFPLTFGGGTKLEIK

SEQ ID NO: 20 - protein, 113 aa, Artificial Sequence
  TRAILshort antibody VL domain
DIVMTQSPDSLAVSLGERATINCKSSQSLLNSGNQKNSLAWYQQRPGHPPKLLLYGASTRESGVPDRFSGSGSGTDFTLTISSLQAEDVAVYYCQNDHSFPLTFGGGTKVEIK

SEQ ID NO: 21 - protein, 113 aa, Artificial Sequence
  TRAILshort antibody VL domain
EIVLTQSPDSLAVSLGERATINCKSSQSLLNSGNQKNSLAWYQHKPGRPPKLLIYGASTRESGVPDRFSGSGSGEDFTLTISSLQAEDVAVYYCQNDHSFPLTFGPGTKVDLK

SEQ ID NO: 22 - protein, 240 aa, Artificial Sequence
  TRAILshort antibody light chain
MVSSAQFLGLLLLCFQGTRCDIVMTQSPSSLSVSAGEKVTMSCKSSQSLLNSGNQKNSLAWYQQKPGRPPTLLISGASTRESGVPDRFTGSGSGTDFTLTISSVQAEDLAVYYCQNDHSFPLTFGAGTKLELKRTVAAPSVFIFPPSDEQLKSGTASVVCLLNNFYPREAKVQWKVDNALQSGNSQESVTEQDSKDSTYSLSSTLTLSKADYEKHKVYACEVTHQGLSSPVTKSFNRGEC

SEQ ID NO: 23 - protein, 240 aa, Artificial Sequence
  TRAILshort antibody light chain
MVSSAQFLGLLLLCFQGTRCDVVMTQSPDSLAVSLGERATINCKSSQSLLNSGNQKNSLAWYQQKPGQPPKLLIYGASTRESGVPDRFSGSGSGTDFTLTISSLQAEDVAVYYCQNDHSFPLTFGQGTKLEIKRTVAAPSVFIFPPSDEQLKSGTASVVCLLNNFYPREAKVQWKVDNALQSGNSQESVTEQDSKDSTYSLSSTLTLSKADYEKHKVYACEVTHQGLSSPVTKSFNRGEC

SEQ ID NO: 24 - protein, 240 aa, Artificial Sequence
  TRAILshort antibody light chain
MVSSAQFLGLLLLCFQGTRCDIVMTQSPDSLAVSLGERATINCKSSQSLLNSGNQKNSLAWYQQKPGQPPKLLIYGASTRESGVPDRFSGSGSGTDFTLTISSLQAEDVAVYYCQNDHSFPLTFGGGTKLEIKRTVAAPSVFIFPPSDEQLKSGTASVVCLLNNFYPREAKVQWKVDNALQSGNSQESVTEQDSKDSTYSLSSTLTLSKADYEKHKVYACEVTHQGLSSPVTKSFNRGEC

SEQ ID NO: 25 - protein, 240 aa, Artificial Sequence
  TRAILshort antibody light chain
MVSSAQFLGLLLLCFQGTRCDIVMTQSPDSLAVSLGERATINCKSSQSLLNSGNQKNSLAWYQQRPGHPPKLLLYGASTRESGVPDRFSGSGSGTDFTLTISSLQAEDVAVYYCQNDHSFPLTFGGGTKVEIKRTVAAPSVFIFPPSDEQLKSGTASVVCLLNNFYPREAKVQWKVDNALQSGNSQESVTEQDSKDSTYSLSSTLTLSKADYEKHKVYACEVTHQGLSSPVTKSFNRGEC

SEQ ID NO: 26 - protein, 240 aa, Artificial Sequence
  TRAILshort antibody light chain
MVSSAQFLGLLLLCFQGTRCEIVLTQSPDSLAVSLGERATINCKSSQSLLNSGNQKNSLAWYQHKPGRPPKLLIYGASTRESGVPDRFSGSGSGEDFTLTISSLQAEDVAVYYCQNDHSFPLTFGPGTKVDLKRTVAAPSVFIFPPSDEQLKSGTASVVCLLNNFYPREAKVQWKVDNALQSGNSQESVTEQDSKDSTYSLSSTLTLSKADYEKHKVYACEVTHQGLSSPVTKSFNRGEC

SEQ ID NO: 27 - protein, 149 aa, Murine
MGWSWIILFLLSGTAGVHCQVQLQQSGPELVKPGASVKISCKASGYIFTNNDMNWVKQRPGQGLEWIGGIDPGDGRTKYNEKFKGKATLTADKFSNTVYMQLSSLTSENSAVYFCGRGGYEFGIDYWGQGTSVTVSSATTTAPSVYPLA

SEQ ID NO: 28 - protein, 163 aa, Murine
MVLMSLLFWVSGTCGDIVMTQSPSSLSVSAGEKVTMSCKSSQSLLNSGNQKNSLAWYQQKPGRPPTLLISGASTRESGVPDRFTGSGSGTDFTLTISSVQAEDLAVYYCQNDHSFPLTFGAGTKLELKRADAAPTVSIFPPSSEQLTSGGASVVCFLNNFYPK

SEQ ID NO: 29 - protein, 330 aa, Homo sapiens [sequence omitted]

SEQ ID NO: 30 - protein, 106 aa, Homo sapiens
TVAAPSVFIFPPSDEQLKSGTASVVCLLNNFYPREAKVQWKVDNALQSGNSQESVTEQDSKDSTYSLSSTLTLSKADYEKHKVYACEVTHQGLSSPVTKSFNRGEC

SEQ ID NO: 31 - DNA, 41 bp, Artificial Sequence
  oligonucleotide probe
tcgttagaaagactccaagaatgaaaaggctctgggccgca